European Patent Application EP 4 306 645 A1, published January 17, 2024. Title: MICROORGANISM OF THE GENUS CORYNEBACTERIUM PRODUCING L-AMINO ACID AND METHOD FOR PRODUCING L-AMINO ACID USING SAME. Applicant: CJ CheilJedang Corporation. The sequence listing filed with the application follows.

SEQUENCE LISTING (8 sequences)

SEQ ID NO: 1 - protein, 344 aa, Artificial Sequence
  NCgl1917
MPNNEFHTNHSLGQDDQTPDQAHFFPQGRGEALVRPGQEHFIAATDETGLGAVDAVADDSAPTSMWGEAWRDLRRRPLFWVSAVLIILALLLAAVPQLFTSTDPQFCVLANSLDGPQSGHPFGFDRQGCDIFARTVYGARASVAVGVLTTLLVALIGTVFGALAGFFGGIMDTILSRITDMFFAIPLVLAAIVVMQMFKEHRTIVTVVLVLGLFGWTNIARITRGAVMTAKNEEYVTSARALGASKAKILLSHIMPNAAAPIIVYATVALGTFIVAEATLSFLGIGLPPSIVSWGADIAKAQTSLRTQPMVLFYPAMALALTVLSFIMMGDVVRDALDPKSRKR

SEQ ID NO: 2 - DNA, 1035 bp, Artificial Sequence
  Ncgl1917
atgcctaataatgaattccacacaaaccactcgttgggccaagatgatcaaaccccagatcaggctcatttcttcccacaaggacgaggcgaggctctagttcgaccaggtcaagagcacttcatcgcagccactgatgaaaccggacttggtgccgtcgatgctgttgctgatgactctgcaccaacctccatgtggggcgaagcgtggcgagaccttcgtcgtcgaccactgttctgggtctctgcggtgttgattattttggcgcttctcctggccgcagttccgcagctgtttacctcaacggatccccagttctgtgtgctggcaaactctcttgatggtccacagtctggacatcccttcggattcgaccgtcaaggttgcgatatttttgctcgtaccgtctacggtgctcgtgcctcggtcgccgtcggtgtgttgaccacgttactggtcgccctcatcggtactgtatttggtgctttggctggcttctttggtggcatcatggataccatcctctcccgcatcaccgacatgttcttcgccattccactggttctggcagccatcgttgtgatgcagatgttcaaggaacaccgcaccatcgtcaccgtggttttggtgcttgggcttttcggctggaccaacattgcgcgtattacccgtggagcggtgatgaccgcaaagaatgaagagtatgtcacctccgcacgtgcgcttggtgcatcaaaagccaagatactgctgtctcacatcatgccaaacgccgcagcacccatcattgtgtatgcaactgtggcactgggaacattcatcgtggcagaggcgacgctctccttcctgggcattggccttccaccatcaattgtctcctggggtgctgatatcgcgaaggcacaaacctcccttcgtacccaacccatggtgctgttctaccccgcaatggcacttgcactaaccgttttgagcttcatcatgatgggcgatgtcgtccgcgacgctctggatcctaagtcgaggaagcgatga

SEQ ID NO: 3 - DNA, 25 bp, Artificial Sequence
  primer
acctacaacaaagctctcatcaacc

SEQ ID NO: 4 - DNA, 24 bp, Artificial Sequence
  primer
ctaccctgtggaacacctacatct

SEQ ID NO: 5 - DNA, 48 bp, Artificial Sequence
  primer
acggccagtgaattcgagctcggtacccatgcctaataatgaattcca

SEQ ID NO: 6 - DNA, 47 bp, Artificial Sequence
  primer
tggtccagccgaaaagcccaagcaccaccgcagagacccagaacagt

SEQ ID NO: 7 - DNA, 20 bp, Artificial Sequence
  primer
gtggtgcttgggcttttcgg

SEQ ID NO: 8 - DNA, 45 bp, Artificial Sequence
  primer
tgcaggtcgactctagaggatcccctcatcgcttcctcgacttag